European Patent Specification EP 3 303 371 B1, published May 3, 2023. Title: Attenuated Bacterium. Applicant: PHARMAQ AS. The sequence listing filed with the application follows.

SEQUENCE LISTING (78 sequences)

SEQ ID NO: 1 - DNA, 1872 bp, Piscirickettsia salmonis
atggatcaacaagaaaaaaggtcgcagtttaaagaactcattgttcgaggtaaacagcaaggctttttaacgtttacagaggtaaacgatcatcttccggatgatatgagcagcccggaagaagttgaagagatcgttgcaatgattagcgacatgggcatccccgtctatgaaactgcacccgatcctgacagcttactcatgaatgagcatgccagctctgccgaagatgatgctgacgatgccgttgcagcgctcgattcagatgctgagtttgggcgaacaaccgacccagtacgcatgtatatgcgcgagatgggcagcgttgagctattaacgcgccaaggtgaaattgagctggctaaacgcatcgaggaaggcgtcaaacaagcctttgaggcaatcgcccattacccacaaagcacagcgattattcttgaagaatatgcaagatttgaagccgaagaaatccgtttagatgatattatcagtggctatatcaccgaagaagatgaagctccgacaagcaacatcggctccatgcttgatgatgccaataaagccgatgataattttgaagccgccttgacagaagacgacagtactgatgacggtgagggtgaggatgacaatgaagaaatccccgtcgataacacattggatgttgaggaagcggcagagcgttttgccgagctaaaagctgcctatgatgcggttatacaggttcaggaaaaacacggaattcatcataaaaaaacacaacagcgttgtgaagaactgtctaaagtattaatgacatttcgcctaaagcccaatatgatcgataaaatcaccaactacttacatggcttactcagccaagtccgcaaacatgagcgtcacatcatggctttgtgcattaatcaagcgaaaatgccccgcaagctatttattgatattttcccaggcaatgaaaccaatctagagtggatagagtatcaaattaaagccgagcaatcttactctgaagcactacagtccctggctccagaagtcactcgtgcacagaaaaagctcatctctcttgaacaagaatcaaactttgatgtcactgcaattaaagaagtcaatcgtaatatttctattggtgaggccaaggcccatcgtgctaaaaaagaaatggtcgaagctaacttgcgtctggtcatctccattgcaaaaaaatacaccaatcgaggcttacaatttctcgacctcattcaagaaggcaatattggcctaatgaaagcggtagataaattcgaataccgccgtggttataaattctcaacgtatgcaacatggtggattcgccaggcaattacccgctcaattgctgatcaagcgcggacaatccggattcctgtacatatgatagagacaattaacaagcttaactgcgtctcacgtcaaatgatccaagaactcggccgtgaagcgactcctgaggagctttctgaacgcatggagatgccagagcataaaatccgtaaaatcctcaaaatcgctaaagagccaatttctatggaaacaccgattggcgatgacgaagattcacacttaggtgattttattgaagataccaccatgcaactccccgttgactcaaccatgggtgatgcgttaaagcaagccaccagtgatattctcgaaaacctcacgccacgtgaagcaaaagtccttagaatgcgctttggtatcgatatgaatactgaccatacgctagaggaagttggcaaacaatttgacgtaactcgcgagcgtattcgccaaattgaagccaaagccttacgtaaactgcgccacccaactcgctcagaaattttgaagagttttcttgactcagaagaataa

SEQ ID NO: 2 - DNA, 20 bp, Artificial Sequence
  PCR Primer: Forward rpoD
ccaggcaattacccgctcaa

SEQ ID NO: 3 - DNA, 20 bp, Artificial Sequence
  PCR primer: Reverse rpoD
tcgccaatcggtgtttccat

SEQ ID NO: 4 - DNA, 657 bp, Piscirickettsia salmonis
atgaaaattaatcatcagcctggcggcataatgttgataatgaataatcatggtgaagtgatgacaagctactcacatatgatgatttttttttcaaattatggcgaaaaagtaaagattgagaatcagcgtatcttaaatgataataaactgctatttagtaatagagtgagtagggtgcgttatcggccttgtcttattattgatgcaaaagatgctttatcagtctgttctggcgtgtttcattaagtaaaaaatgaattcggagttgttgttgcaagctctcttaatgtgatgatatacgattataaatcaatgtcagatgaggatattattcatattttaaagtctgtcaaaaaacatccaaaattatctttaatagaaagcaagatactttttttaaaagtggtaatgaaagggataaaatgtcgccatattgagtcgttacttaaggtatccggaagtactgtgtatacgtattgtatgaatatcaagtcaaaagcaaatatttttagttttaaagggcagtccgtaattcaggaattagaaaaaagtcaattttttagtgatatttctataaagataaatatagatttctataacattaataatggagtaaatgagaaaaatgtttgccaagtatatagcctagcttaa

SEQ ID NO: 5 - DNA, 22 bp, Artificial Sequence
  PCR Primer: Forward FecR
tggtgaagtgatgacaagctac

SEQ ID NO: 6 - DNA, 22 bp, Artificial Sequence
  PCR Primer: Reverse FecR
acacagtacttccggatacctt

SEQ ID NO: 7 - DNA, 951 bp, Piscirickettsia salmonis
atgatcagcctgtggaagacctatcaggcgcttaaaacaaagggcattttaggcattaatcagcgtaatgctgactttattattcgctataatcagcgcaaatactaccctttagtcgatgataaaatcatgacaaaaacccttgcgattaaagatggtattgccgtccctaaattatatgcaacccttaaaactgaccatgatactcaccatctggagcaaattttagccaatcgaacggattttgtcattaaaccggcccgtggtgctggcggtgatggtattttagtcattaccaaccgccatggtgagcgttttcgcaaagtcagtggtgcactgttacacttagacgatattcgtcatcacatttctaatatcttaagtggggtatacagtcttggtggccaacgtgatcaggccatgattgaataccgcgtacaatttgatccattatttaaaaaaatcagctatcaaggtgtgcccgatattcgtattattgtcctaaaaggctatcctgcgatggcgatggtgcgtctacccactcggctccctgatggcaaagccaaccttcatcaaggtgcaattggcgttggcattgacttaacaacaggcatcaccttagaaggtgtttggatgaatgacccaattcatgaacatccggatactggctatgctgtaccaggcttacagattcctcactgggatcattttttaaaccttgctgcacgctgttacgagcttactcaactaggttatttaggtgtggatattatccttgataaagacaaaggcccactcatgcttgagcttaatgcgcgtcctggtttaaatattcaaattgcgaataatagcggcttattgcatcgattacgtttcattgagcaacaaaatcaacaacgcacagccgatgaacgcattgctttcatcaaacatcagttcgcaaaaatataa

SEQ ID NO: 8 - DNA, 20 bp, Artificial Sequence
  PCR Primer: Forward ATP-grasp domain protein
ggtgagcgttttcgcaaagt

SEQ ID NO: 9 - DNA, 20 bp, Artificial Sequence
  PCR Primer: Reverse ATP-grasp domain protein
tcaagcatgagtgggccttt

SEQ ID NO: 10 - DNA, 1983 bp, Piscirickettsia salmonis
atgattaaaaacatcatgctatggctggtcattgctttggtgttggtgactgtgtttagtaatttaggcccacgtcagcagtcggtgaatcggctagattattcaacatttgttaaagacatcaataatggtcaagtaaaaagcgttatcattgatggtttgaatattaaaggacaaacctcaagtgggacgccatttgctacttatattccgtggaaagatccatttttaatggatcagatgctggcgaaaaatgtcacaattgctgctaaaccacctgagcagcggagctggttattgtctgcattaatcagttggttccctggtattttattaattgcgatttggattttcttcttgcggcagatgcaaggcggtggtggtggtaagggcatgatgtcctttggttccagtaaggcacgtctgcttggtgaagatcaaattaaagttaactttgctgatgttgctggctgtgaagaggctaaagaagaagtaaaagaactggtcgattttctgcgtgacccaaccaaattccaaaagttaggcggcaaaattccgcaaggggtattgatagttggcccacctggaacaggtaagacgctattagctaaagccattgcaggtgaggcgaaagtcccgttcttttctatttcaggctctgattttgttgaaatgttcgtcggtgtcggtgcatcgcgggtgcgtgatatgtttgatcaggcaaaaaaacgtgcaccgtgtattatctttatcgatgagattgatgcagtgggccgtcaccgtggctcaggtatgggcggtggtcatgacgaacgtgagcagaccttaaatcaaatgctggtcgagatggatggttttgagggaaccgaaggggtgattgtcattgccgcgacgaatcgtccggatgtattggacccggcattattgcgtcccgggcgttttgatcgccaggtcagtgtcgggcttcccgatgtcaaaggccgtgagcagattctaaaagtgcatatgcgtaaggtgcctttgggagatgatgttaaagcgtcattgatcgcccgtggtacgcctgggttctcaggagcggatttggcgaacttggtcaatgaagccgcactctttgccgcgcgtaaagataaaaccgtggttgctatgcgtgagtttgatgatgccaaagataaaattttgatgggcactgagcgccgttcgatggcaatgaccgaagagcaaaaacgtttaaccgcctttcatgaggcagggcacgcgattgtcgggtgtttggtacctgatcatgatccggtgtataaagtctcgattgtgccgcggggtcgtgccttaggtgtgaccatgtatctgcctgaagaggatagttatggttattcacgcgagcgcttggagagcttaatttcgagtatgtatggcggacgtattgctgaagctttagtctttggtgttgagaaagtaacgactggggcatcgaatgacattgaaaaagcctcagaagtggcgcgcaatatggtgacaaagtgggggctgtctgagcgcttagggccgatattatatggacaagaaggcggtgatccgtttggttatggtgcgggtaaaggcacgccggaattttcagatcaaacctctgttgctattgatgaggaagtacgtcagatcattgatcgtaattatacacgcgctgagagcattctaatcaataatcgggatattcttgatgcgatggcggatgcgttgatggtctatgagacgattgatcgtgaccaagtggctgatctaatggcgcgtcggccggtgaaagcaccgaaagattgggatcagccctctgatgagagtggctcatcagcatctggtgatgagttacaacctcttgatgctaatatcaatactgatattaatgagactaagagcgctgatcaagagacagatcagggcgcgccgtcaccagaaataaagggtaaaccagcggatgatcctacctaa

SEQ ID NO: 11 - DNA, 20 bp, Artificial Sequence
  PCR Primer: Forward FtsH
tggttccagtaaggcacgtc

SEQ ID NO: 12 - DNA, 20 bp, Artificial Sequence
  PCR Primer: Reverse FtsH
acaatcaccccttcggttcc

SEQ ID NO: 13 - protein, 623 aa, Piscirickettsia salmonis
MDQQEKRSQFKELIVRGKQQGFLTFTEVNDHLPDDMSSPEEVEEIVAMISDMGIPVYETAPDPDSLLMNEHASSAEDDADDAVAALDSDAEFGRTTDPVRMYMREMGSVELLTRQGEIELAKRIEEGVKQAFEAIAHYPQSTAIILEEYARFEAEEIRLDDIISGYITEEDEAPTSNIGSMLDDANKADDNFEAALTEDDSTDDGEGEDDNEEIPVDNTLDVEEAAERFAELKAAYDAVIQVQEKHGIHHKKTQQRCEELSKVLMTFRLKPNMIDKITNYLHGLLSQVRKHERHIMALCINQAKMPRKLFIDIFPGNETNLEWIEYQIKAEQSYSEALQSLAPEVTRAQKKLISLEQESNFDVTAIKEVNRNISIGEAKAHRAKKEMVEANLRLVISIAKKYTNRGLQFLDLIQEGNIGLMKAVDKFEYRRGYKFSTYATWWIRQAITRSIADQARTIRIPVHMIETINKLNCVSRQMIQELGREATPEELSERMEMPEHKIRKILKIAKEPISMETPIGDDEDSHLGDFIEDTTMQLPVDSTMGDALKQATSDILENLTPREAKVLRMRFGIDMNTDHTLEEVGKQFDVTRERIRQIEAKALRKLRHPTRSEILKSFLDSEE

SEQ ID NO: 14 - protein, 623 aa, Piscirickettsia salmonis
MDQQEKRSQFKELIVRGKQQGFLTFTEVNDHLPDDMSSPEEVEEIVAMISDMGIPVYETAPDPDSLLMNEHASSAEDDADDAVAALDSDAEFGRTTDPVRMYMREMGSVELLTRQGEIELAKRIEEGVKQAFEAIAHYPQSTAIILEEYARFEAEEIRLDDIISGYITEEDEAPTSNIGSMLDDANKADDNFEAALTEDDSTDDGEGEDDNEEIPVDNTLDVEEAAERFAELKAAYDAVIQVQEKHGIHHKKTQQRCEELSKVLMTFRLKPNMIDKITNYLHGLLSQVRKHERHIMALCINQAKMPRKLFIDIFPGNETNLEWIEYQIKAEQSYSEALQSLAPEVTRAQKKLISLEQESNFDVTAIKEVNRNISIGEAKAHRAKKEMVEANLRLVISIAKKYTNRGLQFLDLIQEGNIGLMKAVDKFEYRRGYKFSTYATWWIRQAITRSIADQARTIRIPVHMIETINKLNRVSRQMIQELGREATPEELSERMEMPEHKIRKILKIAKEPISMETPIGDDEDSHLGDFIEDTTMQLPVDSTMGDALKQATSDILENLTPREAKVLRMRFGIDMNTDHTLEEVGKQFDVTRERIRQIEAKALRKLRHPTRSEILKSFLDSEE

SEQ ID NO: 15 - protein, 623 aa, Piscirickettsia salmonis
MDQQEKKSQFKELIVRGKQQGFLTFTEVNDHLPDDMSSPEEVEEIVAMISDMGIPVYETAPDPDSLLMNEHASSAEDDADDAVAALGSDAEFGRTTDPVRMYMREMGSVELLTRQGEIELAKRIEEGVKQAFEAIAHYPQSTAIILEEYARFEAEEIRLDDIISGYITEEDEAPTSNIGSMLHDANKADDNFEAALTEDDSTDDAEDEGDNEEIPVDNTLDVEEAAERFAELKAAYDAVIQVQEKHGIHHKKTQQRCEELSKVLMTFRLKPNMIDKITNYLHDLLSQVRKHERHIMALCINQAKMPRKLFIDIFPGNETNLDWIEYQIKAEQSYSEALQSLAPEVTRAQKKLISLEQESNFDVTAIKEVNRNISIGEAKAHRAKKEMVEANLRLVISIAKKYTNRGLQFLDLIQEGNIGLMKAVDKFEYRRGYKFSTYATWWIRQAITRSIADQARTIRIPVHMIETINKLNRVSRQMIQELGREATPEELSERMEMPEHKIRKILKIAKEPISMETPIGDDEDSHLGDFIEDTTMQLPVDSTMGDALKQATSDILENLTPREAKVLRMRFGIDMNTDHTLEEVGKQFDVTRERIRQIEAKALRKLRHPTRSEILKSFLDSEE

SEQ ID NO: 16 - protein, 623 aa, Piscirickettsia salmonis; identical to SEQ ID NO: 14

SEQ ID NO: 17 - protein, 623 aa, Piscirickettsia salmonis; identical to SEQ ID NO: 14

SEQ ID NO: 18 - protein, 43 aa, Piscirickettsia salmonis
VHMIETINKLNRVSRQMIQELGREATPEELSERMEMPEHKIRK

SEQ ID NO: 19 - protein, 43 aa, Piscirickettsia salmonis; identical to SEQ ID NO: 18

SEQ ID NO: 20 - protein, 43 aa, Piscirickettsia salmonis; identical to SEQ ID NO: 18

SEQ ID NO: 21 - protein, 43 aa, Piscirickettsia salmonis; identical to SEQ ID NO: 18

SEQ ID NO: 22 - protein, 43 aa, Piscirickettsia salmonis; identical to SEQ ID NO: 18

SEQ ID NO: 23 - protein, 43 aa, Piscirickettsia salmonis; identical to SEQ ID NO: 18

SEQ ID NO: 24 - protein, 43 aa, Piscirickettsia salmonis; identical to SEQ ID NO: 18

SEQ ID NO: 25 - protein, 82 aa, Piscirickettsia salmonis
MKINHQPGGIMLIMNNHGEVMTSYSHMMIFFSNYGEKVKIENQRILNDNKLLFSNRVSRVRYRPCLIIDAKDALSVCSGVFH

SEQ ID NO: 26 - protein, 218 aa, Piscirickettsia salmonis
MKINHQPGGIMLIMNNHGEVMTSYSHMMSFFSNYGEKVKIENQRILNDNKLLFSNRVSRVRYRPCLIIDAKDALSVCSGVFHQVKNEFGVVVASSLNVMIYDYKSMSDEDIIHILKSVKKHPKLSLIESKILFLKVVMKGIKCRHIESLLKVSGSTVYTYCMNIKSKANIFSFKGQSVIQELEKSQFFSDISIKINIDFYNINNGVNEKNVCQVYSLA

SEQ ID NO: 27 - protein, 218 aa, Piscirickettsia salmonis; identical to SEQ ID NO: 26

SEQ ID NO: 28 - protein, 218 aa, Piscirickettsia salmonis
MKINHQPGGIMLIMNNHGEVMTSYSHMMSFFSNYGEKVKIENQRILNDNKLLFSNRVSEVRYRPCLIIDAKDAFSVCSGVFHQVKNEFGVVVANSLNVMIYDYKSMSDEDIIHILKSVKKHPKLSLIESKILFLKVVMKGIKCRHIESLLKVSGSTVYTYCMNIKSKANIFSFKGQSVIQELEKSQFFSDIAMKINIDFYSINNEANEKNVCQVYSLA

SEQ ID NO: 29 - protein, 218 aa, Piscirickettsia salmonis
MKINHQPGGIMLIMNNHGEVMTSYSHMMIFFSNYGEKVKIENQRILNDNKLLFSNRVSRVRYRPCLIIDAKDALSVCSGVFHQVKNEFGVVVASSLNVMIYDYKSMSDEDIIHILKSVKKHPKLSLIESKILFLKVVMKGIKCRHIESLLKVSGSTVYTYCMNIKSKANIFSFKGQSVIQELEKSQFFSDISIKINIDFYNINNGVNEKNVCQVYSLA

SEQ ID NO: 30 - protein, 99 aa, Piscirickettsia salmonis
KIENQRILNDNKLLFSNRVSRVRYRPCLIIDAKDALSVCSGVFHQVKNEFGVVVASSLNVMIYDYKSMSDEDIIHILKSVKKHPKLSLIESKILFLKVV

SEQ ID NO: 31 - protein, 99 aa, Piscirickettsia salmonis; identical to SEQ ID NO: 30

SEQ ID NO: 32 - protein, 99 aa, Piscirickettsia salmonis; identical to SEQ ID NO: 30

SEQ ID NO: 33 - protein, 99 aa, Piscirickettsia salmonis; identical to SEQ ID NO: 30

SEQ ID NO: 34 - protein, 99 aa, Piscirickettsia salmonis
KIENQRILNDNKLLFSNRVSEVRYRPCLIIDAKDAFSVCSGVFHQVKNEFGVVVANSLNVMIYDYKSMSDEDIIHILKSVKKHPKLSLIESKILFLKVV

SEQ ID NO: 35 - protein, 99 aa, Piscirickettsia salmonis; identical to SEQ ID NO: 34

SEQ ID NO: 36 - protein, 99 aa, Piscirickettsia salmonis; identical to SEQ ID NO: 34

SEQ ID NO: 37 - protein, 99 aa, Piscirickettsia salmonis; identical to SEQ ID NO: 34

SEQ ID NO: 38 - protein, 99 aa, Piscirickettsia salmonis; identical to SEQ ID NO: 34

SEQ ID NO: 39 - protein, 316 aa, Piscirickettsia salmonis
MISLWKTYQALKTKGILGINQRNADFIIRYNQRKYYPLVDDKIMTKTLAIKDGIAVPKLYATLKTDHDTHHLEQILANRTDFVIKPARGAGGDGILVITNRHGERFRKVSGALLHLDDIRHHISNILSGVYSLGGQRDQAMIEYRVQFDPLFKKISYQGVPDIRIIVLKGYPAMAMVRLPTRLPDGKANLHQGAIGVGIDLTTGITLEGVWMNDPIHEHPDTGYAVPGLQIPHWDHFLNLAARCYELTQLGYLGVDIILDKDKGPLMLELNARPGLNIQIANNSGLLHRLRFIEQQNQQRTADERIAFIKHQFAKI

SEQ ID NO: 40 - protein, 316 aa, Piscirickettsia salmonis
MISLWKTYQALKTKGILGINQRNADFIIRYNQRKYYPLVDDKIMTKTLAIKDGIAVPKLYATLKTDHDTHHLEQILANRTDFVIKPARGAGGDGILVITNRHGERFRKVSGALLHLDDIRHHISNILSGVYSLGGQRDQAMIEYRVQFDPLFKKISYQGVPDIRIIVLKGYPAMAMVRLPTRLSDGKANLHQGAIGVGIDLTTGITLEGVWMNDPIHEHPDTGYAVPGLQIPHWDHFLNLAARCYELTQLGYLGVDIILDKDKGPLMLELNARPGLNIQIANNSGLLHRLRFIEQQNQQRTADERIAFIKHQFAKI

SEQ ID NO: 41 - protein, 316 aa, Piscirickettsia salmonis; identical to SEQ ID NO: 40

SEQ ID NO: 42 - protein, 316 aa, Piscirickettsia salmonis; identical to SEQ ID NO: 40

SEQ ID NO: 43 - protein, 316 aa, Piscirickettsia salmonis; identical to SEQ ID NO: 40

SEQ ID NO: 44 - protein, 134 aa, Piscirickettsia salmonis
DIRHHISNILSGVYSLGGQRDQAMIEYRVQFDPLFKKISYQGVPDIRIIVLKGYPAMAMVRLPTRLSDGKANLHQGAIGVGIDLTTGITLEGVWMNDPIHEHPDTGYAVPGLQIPHWDHFLNLAARCYELTQLG

SEQ ID NO: 45 - protein, 134 aa, Piscirickettsia salmonis; identical to SEQ ID NO: 44

SEQ ID NO: 46 - protein, 134 aa, Piscirickettsia salmonis; identical to SEQ ID NO: 44

SEQ ID NO: 47 - protein, 134 aa, Piscirickettsia salmonis; identical to SEQ ID NO: 44

SEQ ID NO: 48 - protein, 134 aa, Piscirickettsia salmonis; identical to SEQ ID NO: 44

SEQ ID NO: 49 - protein, 134 aa, Piscirickettsia salmonis; identical to SEQ ID NO: 44

SEQ ID NO: 50 - protein, 134 aa, Piscirickettsia salmonis; identical to SEQ ID NO: 44

SEQ ID NO: 51 - protein, 134 aa, Piscirickettsia salmonis; identical to SEQ ID NO: 44

SEQ ID NO: 52 - protein, 134 aa, Piscirickettsia salmonis; identical to SEQ ID NO: 44

SEQ ID NO: 53 - protein, 660 aa, Piscirickettsia salmonis
MIKNIMLWLVIALVLVTVFSNLGPRQQSVNRLDYSTFVKDINNGQVKSVIIDGLNIKGQTSSGTPFATYIPWKDPFLMDQMLAKNVTIAAKPPEQRSWLLSALISWFPGILLIAIWIFFLRQMQGGGGGKGMMSFGSSKARLLGEDQIKVNFADVAGCEEAKEEVKELVDFLRDPTKFQKLGGKIPQGVLIVGPPGTGKTLLAKAIAGEAKVPFFSISGSDFVEMFVGVGASRVRDMFDQAKKRAPCIIFIDEIDAVGRHRGSGMGGGHDEREQTLNQMLVEMDGFEGTEGVIVIAATNRPDVLDPALLRPGRFDRQVSVGLPDVKGREQILKVHMRKVPLGDDVKASLIARGTPGFSGADLANLVNEAALFAARKDKTVVAMREFDDAKDKILMGTERRSMAMTEEQKRLTAFHEAGHAIVGCLVPDHDPVYKVSIVPRGRALGVTMYLPEEDSYGYSRERLESLISSMYGGRIAEALVFGVEKVTTGASNDIEKASEVARNMVTKWGLSERLGPILYGQEGGDPFGYGAGKGTPEFSDQTSVAIDEEVRQIIDRNYTRAESILINNRDILDAMADALMVYETIDRDQVADLMARRPVKAPKDWDQPSDESGSSASGDELQPLDANINTDINETKSADQETDQGAPSPEIKGKPADDPT

SEQ ID NO: 54 - protein, 660 aa, Piscirickettsia salmonis
MIKNIMLWLVIALVLVTVFSNLGPRQQSVNRLDYSTFVKDINNGQVKSVIIDGLNIKGQTSSGTPFATYIPWKDPFLMDQMLAKNVTIAAKPPEQRSWLLSALISWFPGILLIAIWIFFLRQMQGGGGGKGMMSFGSSKARLLGEDQIKVNFADVAGCEEAKEEVKELVDFLRDPTKFQKLGGKIPQGVLMVGPPGTGKTLLAKAIAGEAKVPFFSISGSDFVEMFVGVGASRVRDMFDQAKKRAPCIIFIDEIDAVGRHRGSGMGGGHDEREQTLNQMLVEMDGFEGTEGVIVIAATNRPDVLDPALLRPGRFDRQVSVGLPDVKGREQILKVHMRKVPLGDDVKASLIARGTPGFSGADLANLVNEAALFAARKDKTVVAMREFDDAKDKILMGTERRSMAMTEEQKRLTAFHEAGHAIVGCLVPDHDPVYKVSIVPRGRALGVTMYLPEEDSYGYSRERLESLISSMYGGRIAEALVFGVEKVTTGASNDIEKASEVARNMVTKWGLSERLGPILYGQEGGDPFGYGAGKGTPEFSDQTSVAIDEEVRQIIDRNYTRAESILINNRDILDAMADALMVYETIDRDQVADLMARRPVKAPKDWDQPSDESGSSASGDELQPLDANINTDINETKSADQETDQGAPSPEIKGKPADDPT

SEQ ID NO: 55 - protein, 660 aa, Piscirickettsia salmonis; identical to SEQ ID NO: 54

SEQ ID NO: 56 - protein, 660 aa, Piscirickettsia salmonis
MIKNIMLWLVIALVLVTVFSNLGPRQQSVNRLDYSTFVKDINNGQVKSVIIDGLNIKGQTSSGTPFATYIPWKDPFLMDQMLSKNVTIAAKPPEQRSWLLSALISWFPGILLIAIWIFFLRQMQGGGGGKGMMSFGSSKARLLGEDQIKVNFADVAGCEEAKEEVKELVDFLRDPTKFQKLGGKIPQGVLMVGPPGTGKTLLAKAIAGEAKVPFFSISGSDFVEMFVGVGASRVRDMFDQAKKRAPCIIFIDEIDAVGRHRGSGMGGGHDEREQTLNQMLVEMDGFEGTEGVIVIAATNRPDVLDPALLRPGRFDRQVSVGLPDVKGREQILKVHMRKVPLGDDVKASLIARGTPGFSGADLANLVNEAALFAARKDKTVVAMREFDDAKDKILMGTERRSMAMTEEQKRLTAFHEAGHAIVGCLVPDHDPVYKVSIVPRGRALGVTMYLPEEDSYGYSRERLESLISSMYGGRIAEALVFGVEKVTTGASNDIEKASEVARNMVTKWGLSERLGPILYGQEGGDPFGYGAGKGTPEFSDQTSVAIDEEVRQIIDRNYTRAESILIDNRDILDAMADALMVYETIDREQVADLMARRPVKAPKDWDQPSDESGSSASGDELQPLDANINTDINDTKSADQEIDQGAPSPEIKGKPADDPT

SEQ ID NO: 57 - protein, 660 aa, Piscirickettsia salmonis; identical to SEQ ID NO: 54

SEQ ID NO: 58 - protein, 123 aa, Piscirickettsia salmonis
FADVAGCEEAKEEVKELVDFLRDPTKFQKLGGKIPQGVLMVGPPGTGKTLLAKAIAGEAKVPFFSISGSDFVEMFVGVGASRVRDMFDQAKKRAPCIIFIDEIDAVGRHRGSGMGGGHDEREQ

SEQ ID NO: 59 - protein, 123 aa, Piscirickettsia salmonis; identical to SEQ ID NO: 58

SEQ ID NO: 60 - protein, 123 aa, Piscirickettsia salmonis; identical to SEQ ID NO: 58

SEQ ID NO: 61 - protein, 123 aa, Piscirickettsia salmonis; identical to SEQ ID NO: 58

SEQ ID NO: 62 - protein, 123 aa, Piscirickettsia salmonis; identical to SEQ ID NO: 58

SEQ ID NO: 63 - protein, 123 aa, Piscirickettsia salmonis; identical to SEQ ID NO: 58

SEQ ID NO: 64 - protein, 123 aa, Piscirickettsia salmonis; identical to SEQ ID NO: 58

SEQ ID NO: 65 - protein, 123 aa, Piscirickettsia salmonis; identical to SEQ ID NO: 58

SEQ ID NO: 66 - protein, 123 aa, Piscirickettsia salmonis; identical to SEQ ID NO: 58

SEQ ID NO: 67 - DNA, 25 bp, Artificial Sequence
  PCR Primer: rpoD SNP Detection Forward Primer
ggacaatccggattcctgtacatat

SEQ ID NO: 68 - DNA, 19 bp, Artificial Sequence
  DNA probe: rpoD VProbe1-VIC Mutant Allele
acaagcttaactgcgtctc

SEQ ID NO: 69 - DNA, 17 bp, Artificial Sequence
  DNA probe: rpoD MProbe2-FAM Wild-Type Allele
aagcttaaccgcgtctc

SEQ ID NO: 70 - DNA, 23 bp, Artificial Sequence
  PCR Primer: rpoD SNP Detection Reverse Primer
gccgagttcttggatcatttgac

SEQ ID NO: 71 - DNA, 18 bp, Artificial Sequence
  PCR Primer: ATP-Grasp Domain Protein SNP Detection Forward Primer
tggcgatggtgcgtctac

SEQ ID NO: 72 - DNA, 16 bp, Artificial Sequence
  DNA probe: ATP-Grasp Domain Protein VProbe1-VIC Mutant Allele
ccatcagggagccgag

SEQ ID NO: 73 - DNA, 16 bp, Artificial Sequence
  DNA probe: ATP-Grasp Domain Protein MProbe2-FAM Wild-Type Allele
ccatcagagagccgag

SEQ ID NO: 74 - DNA, 22 bp, Artificial Sequence
  PCR Primer: ATP-Grasp Domain Protein SNP Detection Reverse Primer
cgccaattgcaccttgatgaag

SEQ ID NO: 75 - DNA, 24 bp, Artificial Sequence
  PCR Primer: FtsH SNP Detection Forward Primer
ccaaaagttaggcggcaaaattcc

SEQ ID NO: 76 - DNA, 14 bp, Artificial Sequence
  DNA probe: FtsH VProbe1-VIC Mutant Allele
tgggccaactatca

SEQ ID NO: 77 - DNA, 14 bp, Artificial Sequence
  DNA probe: FtsH MProbe2-FAM Wild-Type Allele
tgggccaaccatca

SEQ ID NO: 78 - DNA, 24 bp, Artificial Sequence
  PCR Primer: FtsH SNP Detection Reverse Primer
gctaatagcgtcttacctgttcca